European Patent Application EP 4 342 913 A1, published March 27, 2024. Title: CHIMERIC ANTIGEN RECEPTOR MOLECULE FOR SPECIFICALLY RECOGNIZING BAFF-R AND APPLICATION OF CHIMERIC ANTIGEN RECEPTOR MOLECULE. Applicant: Shanghai Escugen Biotechnology Co., Ltd. Guangzhou Yinnuolai Biotechnology Co., Ltd. The sequence listing filed with the application follows.

SEQUENCE LISTING (26 sequences)

SEQ ID NO: 1 - DNA, 63 bp, Artifical sequence
  CD8α signal peptide-encoding nucleotide
atggccctccctgtcaccgccctgctgcttccgctggctcttctgctccacgccgctcggccc

SEQ ID NO: 2 - protein, 21 aa, Artifical sequence
  Human CD8α signal peptide
MALPVTALLLPLALLLHAARP

SEQ ID NO: 3 - DNA, 738 bp, Artifical sequence
  scFv nucleotide sequence
gacatccagatgacacagagccctgatagcctggccgtgtctctgggagagagagccaccatcaactgcaagagcagccagagcgtgctgtactccagcaacaacaagaactacctggcctggtatcagcagaagcccggccagcctcctaagctgctgatctactgggccagcatcagagaaagcggcgtgcccgatagattttccggctctggcagcggcaccgacttcaccctgaccatatctagcctgcagcctgaggacttcgccacctactactgccagcagagctacagcaccccttggacatttggccagggcaccaagctggaaatcaagggaggcggaggttctggcggcggaggaagtggtggcggaggctctgaggttcagctgcaagagtctggccctggcctggtcaagcctagccaaacactgagcctgacctgtaccgtgtccggcgatagcatcacaagcggctactggaactggatcagacagcaccctggcaagggcctcgagtacatcggctacatcagctacagcggcagcacctactacaaccccagcctgaagtccagagtgaccatcagcagagacaccagcaagaaccagtactccctgaagctgagcagcgtgacagccgccgatacagccgtgtactactgcgcctctcctaactaccccttctacgccatggactactggggccagggaaccctggttaccgttagctct

SEQ ID NO: 4 - protein, 246 aa, Artifical sequence
  scFv amino acid sequence
DIQMTQSPDSLAVSLGERATINCKSSQSVLYSSNNKNYLAWYQQKPGQPPKLLIYWASIRESGVPDRFSGSGSGTDFTLTISSLQPEDFATYYCQQSYSTPWTFGQGTKLEIKGGGGSGGGGSGGGGSEVQLQESGPGLVKPSQTLSLTCTVSGDSITSGYWNWIRQHPGKGLEYIGYISYSGSTYYNPSLKSRVTISRDTSKNQYSLKLSSVTAADTAVYYCASPNYPFYAMDYWGQGTLVTVSS

SEQ ID NO: 5 - protein, 118 aa, Artifical sequence
  VH
EVQLQESGPGLVKPSQTLSLTCTVSGDSITSGYWNWIRQHPGKGLEYIGYISYSGSTYYNPSLKSRVTISRDTSKNQYSLKLSSVTAADTAVYYCASPNYPFYAMDYWGQGTLVTVSS

SEQ ID NO: 6 - protein, 5 aa, Artifical sequence
  CDR H1
SGYWN

SEQ ID NO: 7 - protein, 16 aa, Artifical sequence
  CDR H2
YISYSGSTYYNPSLKS

SEQ ID NO: 8 - protein, 10 aa, Artifical sequence
  CDR H3
PNYPFYAMDY

SEQ ID NO: 9 - protein, 113 aa, Artifical sequence
  VL
DIQMTQSPDSLAVSLGERATINCKSSQSVLYSSNNKNYLAWYQQKPGQPPKLLIYWASIRESGVPDRFSGSGSGTDFTLTISSLQPEDFATYYCQQSYSTPWTFGQGTKLEIK

SEQ ID NO: 10 - protein, 17 aa, Artifical sequence
  CDR L1
KSSQSVLYSSNNKNYLA

SEQ ID NO: 11 - protein, 7 aa, Artifical sequence
  CDR L2
WASIRES

SEQ ID NO: 12 - protein, 9 aa, Artifical sequence
  CDR L3
QQSYSTPWT

SEQ ID NO: 13 - DNA, 135 bp, Artifical sequence
  CD8α hinge region nucleotide sequence
accacgacgccagcgccgcgaccaccaacaccggcgcccaccatcgcgtcgcagcccctgtccctgcgcccagaagcgtgccggccagcggcggggggcgcagtgcacacgagggggctggacttcgcctgtgat

SEQ ID NO: 14 - protein, 45 aa, Artifical sequence
  CD8α hinge region amino acid sequence
TTTPAPRPPTPAPTIASQPLSLRPEACRPAAGGAVHTRGLDFACD

SEQ ID NO: 15 - DNA, 72 bp, Artifical sequence
  CD8α TM nucleotide sequence
atctacatttgggcccctctggctggtacttgcggggtcctgctgctttcactcgtgatcactctttactgt

SEQ ID NO: 16 - protein, 24 aa, Artifical sequence
  CD8α TM amino acid sequence
IYIWAPLAGTCGVLLLSLVITLYC

SEQ ID NO: 17 - DNA, 126 bp, Artifical sequence
  4-1BB intracellular region nucleotide sequence
aagcgcggtcggaagaagctgctgtacatctttaagcaacccttcatgaggcctgtgcagactactcaagaggaggacggctgttcatgccggttcccagaggaggaggaaggcggctgcgaactg

SEQ ID NO: 18 - protein, 42 aa, Artifical sequence
  4-1BB intracellular region amino acid sequence
KRGRKKLLYIFKQPFMRPVQTTQEEDGCSCRFPEEEEGGCEL

SEQ ID NO: 19 - DNA, 336 bp, Artifical sequence
  CD3ζ molecule intracellular region nucleotide sequence
cgcgtgaaattcagccgcagcgcagatgctccagcctacaagcaggggcagaaccagctctacaacgaactcaatcttggtcggagagaggagtacgacgtgctggacaagcggagaggacgggacccagaaatgggcgggaagccgcgcagaaagaatccccaagagggcctgtacaacgagctccaaaaggataagatggcagaagcctatagcgagattggtatgaaaggggaacgcagaagaggcaaaggccacgacggactgtaccagggactcagcaccgccaccaaggacacctatgacgctcttcacatgcaggccctgccgcctcgg

SEQ ID NO: 20 - protein, 112 aa, Artifical sequence
  CD3ζ molecule intracellular region amino acid sequence
RVKFSRSADAPAYKQGQNQLYNELNLGRREEYDVLDKRRGRDPEMGGKPRRKNPQEGLYNELQKDKMAEAYSEIGMKGERRRGKGHDGLYQGLSTATKDTYDALHMQALPPR

SEQ ID NO: 21 - DNA, 20 bp, Artifical sequence
  LTR-F
tgacagccgcctagcatttc

SEQ ID NO: 22 - DNA, 24 bp, Artifical sequence
  LTR-R
gctcgatatcagcagttcttgaag

SEQ ID NO: 23 - DNA, 22 bp, Artifical sequence
  LTR probe
cacgtggcccgagagctgcatc

SEQ ID NO: 24 - DNA, 22 bp, Artifical sequence
  ALB-F
gctgtcatctcttgtgggctgt

SEQ ID NO: 25 - DNA, 21 bp, Artifical sequence
  ALB-R
actcatgggagctgctggttc

SEQ ID NO: 26 - DNA, 26 bp, Artifical sequence
  ALB probe
cctgtcatgcccacacaaatctctcc